European Patent Specification EP 3 077 827 B1, published November 1, 2023. Title: Determination of the unbound Free Fatty Acid profiles in biological and industrial specimens. Applicant: Kleinfeld, Alan Marc Huber, Andrew Henry. The sequence listing filed with the application follows.

SEQUENCE LISTING (1 sequence)

SEQ ID NO: 1 - protein, 139 aa, Rattus norvegicus
  MUTAGEN (131)...(131): rat intestinal fatty acid binding protein with Glu 131 to Asp substitution
  VARIANT (131)...(131): COOH-terminal affinity tag comprising Arg 132, Gly 133 and 6 histidines
AFDGTWKVDRNENYEKFMEKMGINVVKRKLGAHDNLKLTITQEGNKFTVKESSNFRNIDVVFELGVDFAYSLADGTELTGTWTMEGNKLVGKFKRVDNGKELIAVREISGNELIQTYTYEGVEAKRIFKKDRGHHHHHH